European Patent Application EP 4 793 280 A1, published August 19, 2026. Title: 一种重组多肽以及制备神经毒素的方法. Applicant: 北京博特维克生物技术有限公司. Application WO. The sequence listing filed with the application follows.

SEQUENCE LISTING (45 sequences)

SEQ ID NO: 1 - protein, 437 aa, Clostridium botulinum
MPFVNKQFNYKDPVNGVDIAYIKIPNAGQMQPVKAFKIHNKIWVIPERDTFTNPEEGDLNPPPEAKQVPVSYYDSTYLSTDNEKDNYLKGVTKLFERIYSTDLGRMLLTSIVRGIPFWGGSTIDTELKVIDTNCINVIQPDGSYRSEELNLVIIGPSADIIQFECKSFGHEVLNLTRNGYGSTQYIRFSPDFTFGFEESLEVDTNPLLGAGKFATDPAVTLAHELIHAGHRLYGIAINPNRVFKVNTNAYYEMSGLEVSFEELRTFGGHDAKFIDSLQENEFRLYYYNKFKDIASTLNKAKSIVGTTASLQYMKNVFKEKYLLSEDTSGKFSVDKLKFDKLYKMLTEIYTEDNFVKFFKVLNRKTYLNFDKAVFKINIVPKVNYTIYDGFNLRNTNLAANFNGQNTEINNMNFTKLKNFTGLFEFYKLLCVRGIITS

SEQ ID NO: 2 - protein, 848 aa, Clostridium botulinum
ALNDLCIKVNNWDLFFSPSEDNFTNDLNKGEEITSDTNIEAAEENISLDLIQQYYLTFNFDNEPENISIENLSSDIIGQLELMPNIERFPNGKKYELDKYTMFHYLRAQEFEHGKSRIALTNSVNEALLNPSRVYTFFSSDYVKKVNKATEAAMFLGWVEQLVYDFTDETSEVSTTDKIADITIIIPYIGPALNIGNMLYKDDFVGALIFSGAVILLEFIPEIAIPVLGTFALVSYIANKVLTVQTIDNALSKRNEKWDEVYKYIVTNWLAKVNTQIDLIRKKMKEALENQAEATKAIINYQYNQYTEEEKNNINFNIDDLSSKLNESINKAMININKFLNQCSVSYLMNSMIPYGVKRLEDFDASLKDALLKYIYDNRGTLIGQVDRLKDKVNNTLSTDIPFQLSKYVDNQRLLSTFTEYIKNIINTSILNLRYESNHLIDLSRYASKINIGSKVNFDPIDKNQIQLFNLESSKIEVILKNAIVYNSMYENFSTSFWIRIPKYFNSISLNNEYTIINCMENNSGWKVSLNYGEIIWTLQDTQEIKQRVVFKYSQMINISDYINRWIFVTITNNRLNNSKIYINGRLIDQKPISNLGNIHASNNIMFKLDGCRDTHRYIWIKYFNLFDKELNEKEIKDLYDNQSNSGILKDFWGDYLQYDKPYYMLNLYDPNKYVDVNNVGIRGYMYLKGPRGSVMTTNIYLNSSLYRGTKFIIKKYASGNKDNIVRNNDRVYINVVVKNKEYRLATNASQAGVEKILSALEIPDVGNLSQVVVMKSKNDQGITNKCKMNLQDNNGNDIGFIGFHQFNNIAKLVASNWYNRQIERSSRTLGCSWEFIPVDDGWGERPL

SEQ ID NO: 3 - protein, 9 aa, Synthetic construct
GTEEAEKLG

SEQ ID NO: 4 - protein, 1315 aa, Synthetic construct
MPFVNKQFNYKDPVNGVDIAYIKIPNAGQMQPVKAFKIHNKIWVIPERDTFTNPEEGDLNPPPEAKQVPVSYYDSTYLSTDNEKDNYLKGVTKLFERIYSTDLGRMLLTSIVRGIPFWGGSTIDTELKVIDTNCINVIQPDGSYRSEELNLVIIGPSADIIQFECKSFGHEVLNLTRNGYGSTQYIRFSPDFTFGFEESLEVDTNPLLGAGKFATDPAVTLAHELIHAGHRLYGIAINPNRVFKVNTNAYYEMSGLEVSFEELRTFGGHDAKFIDSLQENEFRLYYYNKFKDIASTLNKAKSIVGTTASLQYMKNVFKEKYLLSEDTSGKFSVDKLKFDKLYKMLTEIYTEDNFVKFFKVLNRKTYLNFDKAVFKINIVPKVNYTIYDGFNLRNTNLAANFNGQNTEINNMNFTKLKNFTGLFEFYKLLCVRGIITSKRGTEEAEKLGHHHHHHHHGTEEAEKLGKRALNDLCIKVNNWDLFFSPSEDNFTNDLNKGEEITSDTNIEAAEENISLDLIQQYYLTFNFDNEPENISIENLSSDIIGQLELMPNIERFPNGKKYELDKYTMFHYLRAQEFEHGKSRIALTNSVNEALLNPSRVYTFFSSDYVKKVNKATEAAMFLGWVEQLVYDFTDETSEVSTTDKIADITIIIPYIGPALNIGNMLYKDDFVGALIFSGAVILLEFIPEIAIPVLGTFALVSYIANKVLTVQTIDNALSKRNEKWDEVYKYIVTNWLAKVNTQIDLIRKKMKEALENQAEATKAIINYQYNQYTEEEKNNINFNIDDLSSKLNESINKAMININKFLNQCSVSYLMNSMIPYGVKRLEDFDASLKDALLKYIYDNRGTLIGQVDRLKDKVNNTLSTDIPFQLSKYVDNQRLLSTFTEYIKNIINTSILNLRYESNHLIDLSRYASKINIGSKVNFDPIDKNQIQLFNLESSKIEVILKNAIVYNSMYENFSTSFWIRIPKYFNSISLNNEYTIINCMENNSGWKVSLNYGEIIWTLQDTQEIKQRVVFKYSQMINISDYINRWIFVTITNNRLNNSKIYINGRLIDQKPISNLGNIHASNNIMFKLDGCRDTHRYIWIKYFNLFDKELNEKEIKDLYDNQSNSGILKDFWGDYLQYDKPYYMLNLYDPNKYVDVNNVGIRGYMYLKGPRGSVMTTNIYLNSSLYRGTKFIIKKYASGNKDNIVRNNDRVYINVVVKNKEYRLATNASQAGVEKILSALEIPDVGNLSQVVVMKSKNDQGITNKCKMNLQDNNGNDIGFIGFHQFNNIAKLVASNWYNRQIERSSRTLGCSWEFIPVDDGWGERPL

SEQ ID NO: 5 - DNA, 3945 bp, Synthetic construct
  source 1..3945: mol_type = other DNA
atgccgtttgtgaacaaacagttcaactataaagatccggtgaacggtgttgatatcgcctatatcaaaattccgaatgcaggtcagatgcagccggttaaagcctttaaaatccataacaaaatttgggtgattccggaacgtgatacctttaccaatccggaagaaggtgatctgaatccgcctccggaagcaaaacaggttccggttagctattatgatagcacctatctgagcaccgataacgagaaagataactatctgaaaggtgtgaccaaactgtttgaacgcatttatagtaccgatctgggtcgtatgctgctgaccagcattgttcgtggtattccgttttggggtggtagcaccattgataccgaactgaaagttattgacaccaactgcattaatgtgattcagccggatggtagctatcgtagcgaagaactgaatctggttattattggtccgagcgcagatatcattcagtttgaatgtaaaagctttggccacgaagttctgaatctgacccgtaatggttatggtagtacccagtatattcgtttcagtccggattttacctttggctttgaagaaagcctggaagttgatacaaatccgctgttaggtgcaggtaaatttgcaaccgatccggcagttaccctggcacatgaactgattcatgccggtcatcgtctgtatggtattgcaattaatccgaaccgtgtgttcaaagtgaataccaacgcatattatgaaatgagcggtctggaagtgtcatttgaagaactgcgtacctttggtggtcatgatgccaaatttatcgatagcctgcaagaaaatgaatttcgcctgtactactataacaaattcaaggatattgcgagcaccctgaataaagccaaaagcattgttggcaccaccgcaagcctgcagtatatgaaaaatgtgtttaaagaaaaatatctgctgagcgaagataccagcggtaaatttagcgttgacaaactgaaattcgataaactgtacaagatgctgaccgagatttataccgaagataacttcgtgaagtttttcaaagtgctgaaccgcaaaacctacctgaactttgataaagccgtgttcaaaatcaacatcgtgccgaaagtgaactataccatctatgatggttttaacctgcgcaataccaatctggcagcaaactttaatggtcagaacaccgaaatcaacaacatgaactttaccaaactgaagaacttcaccggtctgttcgaattttacaaactgctgtgtgttcgtggcattattaccagcaaacgaggaacagaagaggctgaaaaactagggcaccaccatcatcatcaccaccacggcaccgaagaggcggagaagctgggtaaacgtgccctgaatgatctgtgcattaaggtgaataattgggacctgtttttcagcccgagtgaagataatttcaccaacgatctgaacaaaggcgaagaaattaccagcgataccaatattgaagcagccgaagaaaacattagcctggatctgattcagcagtattatctgaccttcaacttcgataatgagccggaaaatatcagcattgaaaacctgagcagcgatattattggccagctggaactgatgccgaatattgaacgttttccgaacggcaaaaagtacgagctggataaatacaccatgttccattatctgcgtgcccaagaatttgaacatggtaaaagccgtattgcactgaccaatagcgttaatgaagcactgctgaacccgagccgtgtttatacctttttcagcagcgattatgtgaagaaggttaacaaagcaaccgaagcagcaatgtttttaggttgggttgaacagctggtgtatgatttcaccgatgaaaccagcgaagttagcaccaccgataaaattgcagatattaccatcatcatcccgtatatcggtccggcactgaatattggcaatatgctgtataaagacgattttgtgggtgccctgatttttagcggtgcagttattctgctggaatttattccggaaattgccattccggttctgggcacctttgcactggtgagctatattgcaaataaagttctgaccgtgcagaccatcgataatgcactgagcaaacgtaacgaaaaatgggatgaagtgtacaagtatatcgtgaccaattggctggcaaaagttaacacccagattgatctgatccgtaaaaagatgaaagaagccctggaaaatcaggcagaagcaaccaaagccattatcaactatcagtataaccagtacaccgaggaagagaagaataacatcaacttcaacatcgatgatctgagcagcaagctgaatgaaagcatcaacaaagccatgattaacattaacaaatttctgaaccagtgcagcgtgagctatctgatgaatagcatgattccgtatggtgtgaaacgtctggaagattttgatgcaagcctgaaagatgctctgctgaaatatatctatgataatcgtggcaccctgattggtcaggttgatcgtctgaaagataaagtgaacaacaccctgagtaccgatattccttttcagctgagcaaatatgtggataatcagcgtctgctgtcaacctttaccgaatacattaagaacatcatcaacaccagcattctgaacctgcgttatgaaagcaatcatctgatcgatctgtctcgctatgcaagcaaaatcaatataggtagcaaggtgaacttcgacccgattgacaaaaatcagatacagctgtttaatctggaaagcagcaaaatcgaagtgatcctgaaaaacgccattgtgtataacagcatgtatgagaatttctcgaccagcttttggattcgcattccgaaatactttaatagcatcagcctgaacaacgagtacaccattattaactgcatggaaaacaatagcggttggaaagtgagcctgaattatggtgagattatttggaccctgcaggatacccaagaaatcaaacagcgtgtggttttcaaatacagccagatgattaatatcagcgactatatcaaccgctggatttttgtgaccattaccaataatcgcctgaataacagcaagatctatattaacggtcgcctgattgatcagaaaccgattagtaatctgggcaatattcatgcgagcaacaacatcatgtttaaactggatggttgtcgtgatacccatcgttatatttggatcaagtacttcaacctgttcgataaagagctgaacgaaaaagaaattaaagatctgtatgataaccagagcaacagcggtattctgaaggatttttggggagattatctgcagtatgacaaaccgtattatatgctgaacctgtacgacccgaacaaatatgttgatgtgaacaatgtgggtatccgtggctatatgtacctgaaaggtccgcgtggtagcgttatgaccacaaacatttatctgaatagcagcctgtatcgcggaaccaaattcatcattaaaaagtatgccagcggcaacaaggataatattgtgcgtaataatgatcgcgtgtacattaacgttgtggtgaagaataaagaatatcgcctggcaaccaatgcaagccaggcaggcgttgagaaaattctgagcgcactggaaattccggatgttggtaatctgagccaggttgttgtgatgaaaagcaaaaatgatcagggcatcaccaacaagtgcaaaatgaatctgcaggacaataacggcaacgatattggttttattggcttccaccagttcaacaatattgcgaaactggttgcaagcaattggtataatcgtcagattgaacgtagcagtcgtaccctgggttgtagctgggaatttatccctgtggatgatggttggggtgaacgtccgctg

SEQ ID NO: 6 - protein, 8 aa, Synthetic construct
HHHHHHHH

SEQ ID NO: 7 - protein, 14 aa, Synthetic construct
GGSHHHHHHHHGGS

SEQ ID NO: 8 - protein, 17 aa, Synthetic construct
GTEEAEKLGHHHHHHHH

SEQ ID NO: 9 - protein, 17 aa, Synthetic construct
HHHHHHHHGTEEAEKLG

SEQ ID NO: 10 - protein, 46 aa, Synthetic construct
GSGSEEGSGEGTEEAEKLGHHHHHHHHGSGSEEGSGEGTEEAEKLG

SEQ ID NO: 11 - protein, 16 aa, Synthetic construct
DDADHHHHHHHHDDAD

SEQ ID NO: 12 - protein, 22 aa, Synthetic construct
TEDAEKLHHHHHHHHTEDAEKL

SEQ ID NO: 13 - protein, 440 aa, Clostridium botulinum
MPVTINNFNYNDPIDNNNIIMMEPPFARGTGRYYKAFKITDRIWIIPERYTFGYKPEDFNKSSGIFNRDVCEYYDPDYLNTNDKKNIFLQTMIKLFNRIKSKPLGEKLLEMIINGIPYLGDRRVPLEEFNTNIASVTVNKLISNPGEVERKKGIFANLIIFGPGPVLNENETIDIGIQNHFASREGFGGIMQMKFCPEYVSVFNNVQENKGASIFNRRGYFSDPALILMHELIHVLHGLYGIKVDDLPIVPNEKKFFMQSTDAIQAEELYTFGGQDPSIITPSTDKSIYDKVLQNFRGIVDRLNKVLVCISDPNININIYKNKFKDKYKFVEDSEGKYSIDVESFDKLYKSLMFGFTETNIAENYKIKTRASYFSDSLPPVKIKNLLDNEIYTIEEGFNISDKDMEKEYRGQNKAINKQAYEEISKEHLAVYKIQMCKSV

SEQ ID NO: 14 - protein, 850 aa, Clostridium botulinum
APGICIDVDNEDLFFIADKNSFSDDLSKNERIEYNTQSNYIENDFPINELILDTDLISKIELPSENTESLTDFNVDVPVYEKQPAIKKIFTDENTIFQYLYSQTFPLDIRDISLTSSFDDALLFSNKVYSFFSMDYIKTANKVVEAGLFAGWVKQIVNDFVIEANKSNTMDKIADISLIVPYIGLALNVGNETAKGNFENAFEIAGASILLEFIPELLIPVVGAFLLESYIDNKNKIIKTIDNALTKRNEKWSDMYGLIVAQWLSTVNTQFYTIKEGMYKALNYQAQALEEIIKYRYNIYSEKEKSNINIDFNDINSKLNEGINQAIDNINNFINGCSVSYLMKKMIPLAVEKLLDFDNTLKKNLLNYIDENKLYLIGSAEYEKSKVNKYLKTIMPFDLSIYTNDTILIEMFNKYNSEILNNIILNLRYKDNNLIDLSGYGAKVEVYDGVELNDKNQFKLTSSANSKIRVTQNQNIIFNSVFLDFSVSFWIRIPKYKNDGIQNYIHNEYTIINCMKNNSGWKISIRGNRIIWTLIDINGKTKSVFFEYNIREDISEYINRWFFVTITNNLNNAKIYINGKLESNTDIKDIREVIANGEIIFKLDGDIDRTQFIWMKYFSIFNTELSQSNIEERYKIQSYSEYLKDFWGNPLMYNKEYYMFNAGNKNSYIKLKKDSPVGEILTRSKYNQNSKYINYRDLYIGEKFIIRRKSNSQSINDDIVRKEDYIYLDFFNLNQEWRVYTYKYFKKEEEKLFLAPISDSDEFYNTIQIKEYDEQPTYSCQLLFKKDEESTDEIGLIGIHRFYESGIVFEEYKDYFCISKWYLKEVKRKPYNLKLGCNWQFIPKDEGWTE

SEQ ID NO: 15 - protein, 1320 aa, Synthetic construct
MPVTINNFNYNDPIDNNNIIMMEPPFARGTGRYYKAFKITDRIWIIPERYTFGYKPEDFNKSSGIFNRDVCEYYDPDYLNTNDKKNIFLQTMIKLFNRIKSKPLGEKLLEMIINGIPYLGDRRVPLEEFNTNIASVTVNKLISNPGEVERKKGIFANLIIFGPGPVLNENETIDIGIQNHFASREGFGGIMQMKFCPEYVSVFNNVQENKGASIFNRRGYFSDPALILMHELIHVLHGLYGIKVDDLPIVPNEKKFFMQSTDAIQAEELYTFGGQDPSIITPSTDKSIYDKVLQNFRGIVDRLNKVLVCISDPNININIYKNKFKDKYKFVEDSEGKYSIDVESFDKLYKSLMFGFTETNIAENYKIKTRASYFSDSLPPVKIKNLLDNEIYTIEEGFNISDKDMEKEYRGQNKAINKQAYEEISKEHLAVYKIQMCKSVKRGTEEAEKLGHHHHHHHHGTEEAEKLGKRAPGICIDVDNEDLFFIADKNSFSDDLSKNERIEYNTQSNYIENDFPINELILDTDLISKIELPSENTESLTDFNVDVPVYEKQPAIKKIFTDENTIFQYLYSQTFPLDIRDISLTSSFDDALLFSNKVYSFFSMDYIKTANKVVEAGLFAGWVKQIVNDFVIEANKSNTMDKIADISLIVPYIGLALNVGNETAKGNFENAFEIAGASILLEFIPELLIPVVGAFLLESYIDNKNKIIKTIDNALTKRNEKWSDMYGLIVAQWLSTVNTQFYTIKEGMYKALNYQAQALEEIIKYRYNIYSEKEKSNINIDFNDINSKLNEGINQAIDNINNFINGCSVSYLMKKMIPLAVEKLLDFDNTLKKNLLNYIDENKLYLIGSAEYEKSKVNKYLKTIMPFDLSIYTNDTILIEMFNKYNSEILNNIILNLRYKDNNLIDLSGYGAKVEVYDGVELNDKNQFKLTSSANSKIRVTQNQNIIFNSVFLDFSVSFWIRIPKYKNDGIQNYIHNEYTIINCMKNNSGWKISIRGNRIIWTLIDINGKTKSVFFEYNIREDISEYINRWFFVTITNNLNNAKIYINGKLESNTDIKDIREVIANGEIIFKLDGDIDRTQFIWMKYFSIFNTELSQSNIEERYKIQSYSEYLKDFWGNPLMYNKEYYMFNAGNKNSYIKLKKDSPVGEILTRSKYNQNSKYINYRDLYIGEKFIIRRKSNSQSINDDIVRKEDYIYLDFFNLNQEWRVYTYKYFKKEEEKLFLAPISDSDEFYNTIQIKEYDEQPTYSCQLLFKKDEESTDEIGLIGIHRFYESGIVFEEYKDYFCISKWYLKEVKRKPYNLKLGCNWQFIPKDEGWTE

SEQ ID NO: 16 - DNA, 3960 bp, Synthetic construct
  source 1..3960: mol_type = other DNA
atgcccgtaacaataaataactttaattataatgacccgattgataacaacaatatcattatgatggaaccgccatttgcgcgtggtactggtcgttattacaaggccttcaaaatcaccgaccgtatttggattattccggaacgttacaccttcggttataagccggaggacttcaataaaagcagcggtattttcaaccgtgatgtgtgtgaatactacgacccggattatctgaatacgaatgacaaaaagaacattttcctgcagacgatgattaagctgtttaaccgcattaaatccaaaccgctgggtgaaaagttgctggagatgatcattaacggtattccgtaccttggagatcgccgtgttccgctggaggaattcaataccaatatcgcgtccgttaccgttaataagttgatcagcaatccgggggaagtggagcgcaaaaaaggtattttcgctaacctgataatcttcggcccaggtccggtgctgaacgagaatgaaaccattgacatcggcattcagaaccactttgcgtctagagaaggatttggcggtatcatgcagatgaaattctgcccggaatacgtgtctgtcttcaataacgtgcaggaaaacaagggtgccagcatcttcaaccgtcgcggttatttcagcgacccggcgctgattctgatgcatgaactcattcatgttctgcatggtttgtacggcatcaaggtagacgatctaccgatcgtgccgaatgaaaagaaattcttcatgcagagcaccgatgcgattcaggccgaagagttgtacacctttggtggtcaagatccgtccatcatcaccccgagcacggacaagtcgatctacgataaagtgctgcaaaactttcgtggcatcgttgaccgcctgaacaaggtgctggtttgcattagcgacccgaatatcaacatcaacatttacaagaataagttcaaggacaagtacaagttcgtcgaagattccgagggtaaatactctatcgacgtcgagagcttcgataaactgtacaagtctctgatgttcggttttaccgaaaccaacatcgcggaaaattacaagattaagacccgtgctagctacttctctgacagcctgccgcctgtgaaaatcaaaaacttgctggacaacgaaatctataccattgaggaaggatttaatatttccgataaagatatggagaaggagtaccgtggccaaaacaaagcgatcaataaacaggcctatgaagagatcagcaaagaacatctggcagtttataagatacagatgtgcaaaagtgtgaagcgcggtaccgaagaggccgagaagttgggccaccatcatcaccaccaccaccacggcaccgaagaggcggaaaagttgggtaaacgcgcgccaggtatttgcatcgatgttgataacgaggatctgtttttcatagcggataaaaatagcttcagcgacgatctgagcaagaatgaacgtatcgagtataacacgcagagcaactatattgagaacgacttcccgattaacgagttaatcctggacaccgacctcatctccaagatcgaattaccgagcgagaatactgagagcctaactgattttaacgtggatgttccggtatatgagaagcaaccggcaattaagaagatcttcaccgacgagaacaccattttccagtatctttacagccaaacgtttccgctcgatatccgtgatatctctctgaccagcagctttgacgacgcgctgctgttctcgaacaaggtttacagctttttcagcatggattacatcaagactgcgaacaaggtcgtcgaggcaggccttttcgcgggctgggttaagcagatcgtgaatgacttcgtcatcgaagcgaacaagtccaacaccatggacaagatcgcggatatttctctcatcgtaccgtacatcggcctggcgctgaatgttggcaatgaaacggctaaaggcaacttcgaaaacgcttttgagatcgccggtgcttcaattctgttagaatttattccggaactgctgatcccggtggttggcgcatttctgttggagagctacatcgacaacaaaaacaagatcattaagacgatcgacaacgctctgaccaagcgtaatgaaaagtggtcggatatgtatggcttgattgtggcccaatggctgagcaccgtgaacacgcaattttatacgattaaggaaggtatgtacaaagcactgaactaccaggcgcaggctttagaagagattatcaaataccgctacaacatttacagcgaaaaggagaagtccaacatcaacatcgactttaacgacattaacagcaagttgaacgagggcatcaatcaagccattgataacattaataactttatcaacggctgtagcgttagctacctgatgaaaaaaatgatcccgctggcagttgagaagctgttggatttcgataacacccttaagaagaatttactgaactacattgatgagaacaagctgtatttaattggtagcgctgaatatgaaaaatctaaagtgaataagtatttaaagaccattatgccttttgacctgagcatctataccaatgacaccatattgattgagatgtttaacaagtacaacagcgaaatcctgaataacataattctgaacctgcgttacaaagacaacaatctcatcgacctgtctggctatggtgcgaaagtcgaggtttacgacggtgttgagctgaatgacaagaaccaatttaagttaacaagcagtgcaaacagcaagatccgcgtgacgcaaaatcaaaatattatttttaactctgtttttctggatttctctgtttccttctggatccgtattccgaaatacaaaaacgacggcattcagaactatatccacaatgaatacacgatcattaactgcatgaaaaataacagcggttggaaaatctcaatccgtggcaatcgtattatctggaccctgatcgatatcaacggcaaaacaaaatccgtgttctttgaatataacattcgcgaagatatctcagagtatatcaaccgttggttctttgtgacgataaccaataacttaaacaacgcgaaaatctatatcaacggtaaacttgagagcaacaccgacattaaagacatccgcgaagttatcgcgaacggtgagattattttcaaattggacggtgatatcgaccgcacccaattcatttggatgaaatatttctccatcttcaacaccgagctgtcccaatcgaacattgaggaacgttataagatccagagctactcggagtacctgaaagacttctggggtaacccgctgatgtataacaaagagtattacatgtttaacgcgggcaacaagaacagctacatcaaattgaaaaaagattccccggttggtgaaattctcacccgttcgaaatacaatcagaatagcaagtatattaattatagagacctgtatattggcgagaagtttatcatccgtagaaagtctaacagccagagcattaatgatgatatcgttcgtaaagaggattatatctacttggattttttcaatctgaaccaagaatggcgtgtgtacacgtacaagtacttcaaaaaggaggaagagaagttattcttggcaccgatcagcgactccgacgagttctataataccattcaaatcaaggagtatgacgagcagccaacttattcctgtcagctgttgtttaaaaaagatgaagagagtaccgacgaaattggtctgatcggcatccaccgtttttatgagtccggcattgtgttcgaagagtacaaggattacttttgcataagcaaatggtatctgaaagaggtgaagcgtaaaccgtacaacctgaaattgggctgcaactggcagtttatccccaaagatgagggatggaccgag

SEQ ID NO: 17 - protein, 416 aa, Clostridium botulinum
MPKINSFNYNDPVNDRTILYIKPGGCQEFYKSFNIMKNIWIIPERNVIGTTPQDFHPPTSLKNGDSSYYDPNYLQSDEEKDRFLKIVTKIFNRINNNLSGGILLEELSKANPYLGNDNTPDNQFHIGDASAVEIKFSNGSQDILLPNVIIMGAEPDLFETNSSNISLRNNYMPSNHRFGSIAIVTFSPEYSFRFNDNCMNEFIQDPALTLMHELIHSLHGLYGAKGITTKYTITQKQNPLITNIRGTNIEEFLTFGGTDLNIITSAQSNDIYTNLLADYKKIASKLSKVQVSNPLLNPYKDVFEAKYGLDKDASGIYSVNINKFNDIFKKLYSFTEFDLRTKFQVKCRQTYIGQYKYFKLSNLLNDSIYNISEGYNINNLKVNFRGQNANLNPRIITPITGRGLVKKIIRFCKNIV

SEQ ID NO: 18 - protein, 828 aa, Clostridium botulinum
SICIEINNGELFFVASENSYNDDNINTPKEIDDTVTSNNNYENDLDQVILNFNSESAPGLSDEKLNLTIQNDAYIPKYDSNGTSDIEQHDVNELNVFFYLDAQKVPEGENNVNLTSSIDTALLEQPKIYTFFSSEFINNVNKPVQAALFVSWIQQVLVDFTTEANQKSTVDKIADISIVVPYIGLALNIGNEAQKGNFKDALELLGAGILLEFEPELLIPTILVFTIKSFLGSSDNKNKVIKAINNALKERDEKWKEVYSFIVSNWMTKINTQFNKRKEQMYQALQNQVNAIKTIIESKYNSYTLEEKNELTNKYDIKQIENELNQKVSIAMNNIDRFLTESSISYLMKIINEVKINKLREYDENVKTYLLNYIIQHGSILGESQQELNSMVTDTLNNSIPFKLSSYTDDKILISYFNKFFKRIKSSSVLNMRYKNDKYVDTSGYDSNININGDVYKYPTNKNQFGIYNDKLSEVNISQNDYIIYDNKYKNFSISFWVRIPNYDNKIVNVNNEYTIINCMRDNNSGWKVSLNHNEIIWTFEDNRGINQKLAFNYGNANGISDYINKWIFVTITNDRLGDSKLYINGNLIDQKSILNLGNIHVSDNILFKIVNCSYTRYIGIRYFNIFDKELDETEIQTLYSNEPNTNILKDFWGNYLLYDKEYYLLNVLKPNNFIDRRKDSTLSINNIRSTILLANRLYSGIKVKIQRVNNSSTNDNLVRKNDQVYINFVASKTHLFPLYADTATTNKEKTIKISSSGNRFNQVVVMNSVGNCTMNFKNNNGNNIGLLGFKADTVVASTWYYTHMRDHTNSNGCFWNFISEEHGWQEK

SEQ ID NO: 19 - protein, 1274 aa, Synthetic construct
MPKINSFNYNDPVNDRTILYIKPGGCQEFYKSFNIMKNIWIIPERNVIGTTPQDFHPPTSLKNGDSSYYDPNYLQSDEEKDRFLKIVTKIFNRINNNLSGGILLEELSKANPYLGNDNTPDNQFHIGDASAVEIKFSNGSQDILLPNVIIMGAEPDLFETNSSNISLRNNYMPSNHRFGSIAIVTFSPEYSFRFNDNCMNEFIQDPALTLMHELIHSLHGLYGAKGITTKYTITQKQNPLITNIRGTNIEEFLTFGGTDLNIITSAQSNDIYTNLLADYKKIASKLSKVQVSNPLLNPYKDVFEAKYGLDKDASGIYSVNINKFNDIFKKLYSFTEFDLRTKFQVKCRQTYIGQYKYFKLSNLLNDSIYNISEGYNINNLKVNFRGQNANLNPRIITPITGRGLVKKIIRFCKNIVKRGTEEAEKLGHHHHHHHHGTEEAEKLGKRSICIEINNGELFFVASENSYNDDNINTPKEIDDTVTSNNNYENDLDQVILNFNSESAPGLSDEKLNLTIQNDAYIPKYDSNGTSDIEQHDVNELNVFFYLDAQKVPEGENNVNLTSSIDTALLEQPKIYTFFSSEFINNVNKPVQAALFVSWIQQVLVDFTTEANQKSTVDKIADISIVVPYIGLALNIGNEAQKGNFKDALELLGAGILLEFEPELLIPTILVFTIKSFLGSSDNKNKVIKAINNALKERDEKWKEVYSFIVSNWMTKINTQFNKRKEQMYQALQNQVNAIKTIIESKYNSYTLEEKNELTNKYDIKQIENELNQKVSIAMNNIDRFLTESSISYLMKIINEVKINKLREYDENVKTYLLNYIIQHGSILGESQQELNSMVTDTLNNSIPFKLSSYTDDKILISYFNKFFKRIKSSSVLNMRYKNDKYVDTSGYDSNININGDVYKYPTNKNQFGIYNDKLSEVNISQNDYIIYDNKYKNFSISFWVRIPNYDNKIVNVNNEYTIINCMRDNNSGWKVSLNHNEIIWTFEDNRGINQKLAFNYGNANGISDYINKWIFVTITNDRLGDSKLYINGNLIDQKSILNLGNIHVSDNILFKIVNCSYTRYIGIRYFNIFDKELDETEIQTLYSNEPNTNILKDFWGNYLLYDKEYYLLNVLKPNNFIDRRKDSTLSINNIRSTILLANRLYSGIKVKIQRVNNSSTNDNLVRKNDQVYINFVASKTHLFPLYADTATTNKEKTIKISSSGNRFNQVVVMNSVGNCTMNFKNNNGNNIGLLGFKADTVVASTWYYTHMRDHTNSNGCFWNFISEEHGWQEK

SEQ ID NO: 20 - DNA, 3822 bp, Synthetic construct
  source 1..3822: mol_type = other DNA
atgcccaaaataaattcatttaattataacgacccagttaatgaccgcacgatcttgtacattaagccgggtggctgccaggaattctataagtcctttaatataatgaaaaacatttggatcatcccggaacgtaatgtcattggcactacgccgcaggacttccatccgccaaccagcctcaagaatggtgactctagctactacgacccgaattacctgcaaagcgacgaggaaaaggacagatttctgaaaattgtgaccaaaatttttaaccgcattaacaacaacctatcgggcggcatcttgcttgaagaattaagcaaggcgaacccttatctgggtaacgacaacaccccagataatcaatttcatattggtgacgcgagcgctgtggaaattaagtttagcaatggctctcaggacattcttctgccgaacgtcatcatcatgggtgcagaaccggatctgtttgagacaaacagctccaacatttctctgcgtaacaactatatgccgagcaaccatcgtttcggtagcatcgcgattgtgaccttttccccggagtacagcttccgcttcaatgacaactgcatgaacgagttcatccaagatccggcactgactctgatgcatgaattaatccacagcctgcatggtttatacggcgctaaaggcattaccaccaaatataccatcacccagaagcaaaacccactgattacgaacatacgtggtacgaacatcgaggagttcctgacgttcggcggtacggatctaaatatcattaccagtgcgcaaagcaacgacatctacacgaatttactcgcggattacaaaaaaatcgccagcaaactttcgaaggtgcaggtgagcaatccgctgctgaacccgtataaagatgtttttgaggcgaaatacggtctggataaagacgccagcggtatttacagcgtcaatattaacaaattcaatgacatcttcaaaaagctgtactccttcaccgagttcgatctgcgtaccaagttccaggttaagtgccgtcaaacctacattggtcaatataagtacttcaagctcagcaatctgctgaacgactcaatttataatatcagcgaaggttataacatcaacaacctgaaagtcaacttccgtggtcagaacgcgaacctaaatccgcgtattattaccccaatcaccggccgtggtctggttaaaaagattattcgtttctgcaaaaacattgttaaaagaggcaccgaggaggcggaaaaattgggccatcaccaccaccaccaccaccacgggaccgaggaagcggaaaagctgggaaaacgtagtatttgtattgaaatcaacaacggcgaactgttcttcgtggctagcgaaaacagctataacgacgacaatattaacactccgaaagagattgacgacaccgtcacctcaaacaataactatgaaaatgacctggatcaggtgattttgaactttaacagcgaatctgcaccgggtctgtccgacgagaaactgaacctgaccatccaaaacgacgcgtatatcccgaaatatgacagcaatggtacgtccgacatcgaacagcatgatgtgaacgagctgaacgtttttttctaccttgatgcccaaaaggtgccggagggtgaaaacaatgttaatctgaccagcagcatcgataccgcactgctggagcagccgaagatttatactttcttcagctccgaattcattaacaacgtgaacaagccggttcaggcggcactgttcgtttcttggattcagcaggttctggttgactttaccaccgaagcgaatcagaagtctacggtcgataaaatcgctgacatctctattgtggtcccgtatatcggcttggcccttaacattggcaacgaagcgcagaagggcaacttcaaggacgcattggagttgctgggtgcgggtatcctattagagttcgagccggagctgttgatcccgaccatcttggtttttaccattaagagcttcctgggtagctcagacaacaagaacaaggttatcaaagcgattaataacgcactgaaggagcgcgatgagaaatggaaagaagtttatagttttatcgtgagcaactggatgaccaaaatcaacacccaatttaataaacgcaaagagcagatgtatcaggctctgcagaaccaggtaaatgccatcaagacgattatcgagagcaaatataacagctacacgctggaggaaaagaacgaactgaccaacaagtacgacatcaaacagattgagaatgagctgaatcagaaagtatctatcgctatgaataacatcgatcgttttctgacggaaagctcgatttcgtaccttatgaaaatcatcaatgaggttaaaatcaataagcttcgtgaatacgatgagaacgtcaaaacctatctgctgaattacatcattcagcacggctctatcctgggcgaatctcagcaagagctgaacagcatggttactgacaccctgaacaacagcatcccgttcaagttgtcctcctacaccgatgacaaaattttgatctcctatttcaataagttcttcaagcgcataaagtccagctccgttttgaacatgcgctacaagaacgacaagtacgtggacactagcggttatgatagcaacatcaatatcaatggcgatgtctataagtacccgaccaacaagaatcaatttggcatttacaatgacaaattgtctgaggtgaacatttctcaaaacgactacattatctatgataataagtacaagaacttttccatttcgttctgggtacgtattcccaactatgataataagatcgttaacgttaataatgagtacaccattatcaactgtatgcgcgataacaacagcggttggaaagtttctctgaaccacaacgaaattatctggaccttcgaagataatcgtggcatcaaccaaaagttggcgtttaactacggtaacgcgaatggcatctctgattatatcaataaatggatctttgtgaccattacgaacgatcgcctgggcgattcgaagttgtacatcaatggcaacctcatcgatcagaagagcatcctgaacttgggcaacattcacgtgagcgacaacatcctgttcaagatcgtgaactgcagctacacccgttatatcggtattcgctattttaacatctttgataaagaactggatgagacagagatccagaccctgtatagcaacgaaccgaataccaatatcctgaaggatttttggggtaattacttgctgtacgacaaagaatactacctgctgaacgtgttgaagccgaacaacttcatcgacagacgtaaagatagcaccttgagtataaacaatatccgctcaactatcctgctggctaaccgtctgtactccggtattaaagtcaaaattcagcgtgttaacaactcgtcaacaaacgacaacctggttcgtaagaacgaccaagtgtacatcaattttgttgcttccaaaacccacctgttcccgctgtatgcagatactgcgaccaccaacaaggagaagacgatcaaaatctctagcagcggcaaccgtttcaaccaagtggtggtgatgaacagcgtgggtaattgcaccatgaatttcaagaacaataatggtaataacatcggtctgttgggctttaaagcggataccgttgtagccagcacctggtattacacccatatgcgtgatcataccaactctaacggctgtttttggaattttatttcggaagagcacggttggcaagaaaaa

SEQ ID NO: 21 - protein, 4 aa, Synthetic construct
GSGS

SEQ ID NO: 22 - protein, 6 aa, Synthetic construct
EEGSGS

SEQ ID NO: 23 - protein, 10 aa, Synthetic construct
GSGSDDGSGS

SEQ ID NO: 24 - protein, 10 aa, Synthetic construct
GSGSEDGSGS

SEQ ID NO: 25 - protein, 10 aa, Synthetic construct
GSGSDEGSGS

SEQ ID NO: 26 - protein, 4 aa, Synthetic construct
EEAE

SEQ ID NO: 27 - protein, 4 aa, Synthetic construct
DDAD

SEQ ID NO: 28 - protein, 7 aa, Synthetic construct
TEEAEKL

SEQ ID NO: 29 - protein, 7 aa, Synthetic construct
TDDADKL

SEQ ID NO: 30 - protein, 7 aa, Synthetic construct
TEDAEKL

SEQ ID NO: 31 - protein, 7 aa, Synthetic construct
TDEADKL

SEQ ID NO: 32 - protein, 9 aa, Synthetic construct
GTEEAEKLG

SEQ ID NO: 33 - protein, 10 aa, Synthetic construct
EGTEEAEKLG

SEQ ID NO: 34 - protein, 10 aa, Synthetic construct
EGTDDADKLG

SEQ ID NO: 35 - protein, 10 aa, Synthetic construct
EGTEEADKLG

SEQ ID NO: 36 - protein, 10 aa, Synthetic construct
EGTDDAEKLG

SEQ ID NO: 37 - protein, 10 aa, Synthetic construct
EGTEDADKLG

SEQ ID NO: 38 - protein, 10 aa, Synthetic construct
EGTDEAEKLG

SEQ ID NO: 39-44 - skipped (6 entries)

SEQ ID NO: 45 - protein, 5 aa, Synthetic construct
DDDDK